European Patent Application EP 4 623 920 A1, published October 1, 2025. Title: A PHARMACEUTICAL COMPOSITION FOR PREVENTING OR TREATING SECONDARY ATROPHIC RHINITIS COMPRISING NASAL TURBINATE-DERIVED STEM CELLS AS AN ACTIVE INGREDIENT. Applicant: 가톨릭대학교 산학협력단. Application EP. The sequence listing filed with the application follows.

SEQUENCE LISTING (10 sequences)

SEQ ID NO: 1 - DNA, 20 bp, synthetic construct
  source 1..20: mol_type = other DNA
gaccagtcaacaggggacat

SEQ ID NO: 2 - DNA, 20 bp, synthetic construct
  source 1..20: mol_type = other DNA
cttgcgaccttgaccatctt

SEQ ID NO: 3 - DNA, 18 bp, synthetic construct
  source 1..18: mol_type = other DNA
tcgactgggaagccatct

SEQ ID NO: 4 - DNA, 19 bp, synthetic construct
  source 1..19: mol_type = other DNA
gtcgaagtccaggctgttg

SEQ ID NO: 5 - DNA, 20 bp, synthetic construct
  source 1..20: mol_type = other DNA
gaaggaggaactggcctacc

SEQ ID NO: 6 - DNA, 20 bp, synthetic construct
  source 1..20: mol_type = other DNA
tctcgtactggtcacgcatc

SEQ ID NO: 7 - DNA, 21 bp, synthetic construct
  source 1..21: mol_type = other DNA
tctgctgtcccgagagaacac

SEQ ID NO: 8 - DNA, 20 bp, synthetic construct
  source 1..20: mol_type = other DNA
ctgccatcacaaatgaccac

SEQ ID NO: 9 - DNA, 20 bp, synthetic construct
  source 1..20: mol_type = other DNA
gcctacagaacccaactgga

SEQ ID NO: 10 - DNA, 20 bp, synthetic construct
  source 1..20: mol_type = other DNA
tctctccgctgtgaatcctt